European Patent Application EP 4 428 234 A2, published September 11, 2024. Title: DIRECT-TO-LIBRARY METHODS, SYSTEMS, AND COMPOSITIONS. Applicant: KARIUS, INC. Application EP. The sequence listing filed with the application follows.

SEQUENCE LISTING (18 sequences)

SEQ ID NO: 1 - DNA, 10 bp, synthetic construct
  misc_feature 1..10: note = Description of Artificial Sequence: Synthetic oligonucleotide
  source 1..10: mol_type = other DNA
agatcggaag

SEQ ID NO: 2 - DNA, 16 bp, synthetic construct
  misc_feature 1..16: note = Description of Artificial Sequence: Synthetic oligonucleotide
  misc_difference 11..16: note = a, c, t, g, unknown or other
  source 1..16: mol_type = other DNA
cttccgatctnnnnnn

SEQ ID NO: 3 - DNA, 16 bp, synthetic construct
  misc_feature 1..16: note = Description of Artificial Sequence: Synthetic oligonucleotide
  misc_difference 11..16: note = a, c, t, g, unknown or other
  source 1..16: mol_type = other DNA
cttccgatctnnnnnn

SEQ ID NO: 4 - DNA, 26 bp, synthetic construct
  misc_feature 1..26: note = Description of Artificial Sequence: Synthetic oligonucleotide
  misc_difference 11..16: note = a, c, t, g, unknown or other
  source 1..26: mol_type = other DNA
cttccgatctnnnnnnagatcggaag

SEQ ID NO: 5 - DNA, 16 bp, synthetic construct
  misc_feature 1..16: note = Description of Artificial Sequence: Synthetic oligonucleotide
  misc_difference 11..16: note = a, c, t, g, unknown or other
  source 1..16: mol_type = other DNA
cttccgatctnnnnnn

SEQ ID NO: 6 - DNA, 50 bp, synthetic construct
  misc_feature 1..50: note = Description of Artificial Sequence: Synthetic oligonucleotide
  source 1..50: mol_type = other DNA
ggcctcgcggaggcatgcgtcatgctagcgtgcggggtactcttgctatc

SEQ ID NO: 7 - DNA, 50 bp, synthetic construct
  misc_feature 1..50: note = Description of Artificial Sequence: Synthetic oligonucleotide
  source 1..50: mol_type = other DNA
gagaattattcgggggcagtgacaaccaacatctcgggtcctgcccaacc

SEQ ID NO: 8 - DNA, 50 bp, synthetic construct
  misc_feature 1..50: note = Description of Artificial Sequence: Synthetic oligonucleotide
  source 1..50: mol_type = other DNA
ggtctacacgctaatatagcgaatcaccgagaacccggcgccacgcaatg

SEQ ID NO: 9 - DNA, 50 bp, synthetic construct
  misc_feature 1..50: note = Description of Artificial Sequence: Synthetic oligonucleotide
  source 1..50: mol_type = other DNA
gaacgtccttaactccggcaggcaattaaagggaacgtatgtataacgca

SEQ ID NO: 10 - DNA, 60 bp, synthetic construct
  misc_feature 1..60: note = Description of Artificial Sequence: Synthetic oligonucleotide
  source 1..60: mol_type = other DNA
atgacgcgctttcaagcgtggcgagtatgtgaaccaaggcttcggacaggagatcggaag

SEQ ID NO: 11 - DNA, 50 bp, synthetic construct
  misc_feature 1..50: note = Description of Artificial Sequence: Synthetic oligonucleotide
  source 1..50: mol_type = other DNA
actatatacttaggtttgatctcgccccgagaactgtaaacctcaacatt

SEQ ID NO: 12 - DNA, 50 bp, synthetic construct
  misc_feature 1..50: note = Description of Artificial Sequence: Synthetic oligonucleotide
  source 1..50: mol_type = other DNA
tgaaatatcttaggtttgatctcgccccgagaactgtaaacctcaacatt

SEQ ID NO: 13 - DNA, 25 bp, synthetic construct
  misc_feature 1..25: note = Description of Artificial Sequence: Synthetic oligonucleotide
  source 1..25: mol_type = other DNA
ttttttttttttttttttttttttt

SEQ ID NO: 14 - DNA, 12 bp, synthetic construct
  misc_feature 1..12: note = Description of Artificial Sequence: Synthetic oligonucleotide
  source 1..12: mol_type = other DNA
cgacgctcttcc

SEQ ID NO: 15 - DNA, 29 bp, synthetic construct
  misc_feature 1..29: note = Description of Artificial Sequence: Synthetic oligonucleotide
  source 1..29: mol_type = other DNA
ggaagagcgtcgtgtagggaaagagtgta

SEQ ID NO: 16 - DNA, 34 bp, synthetic construct
  misc_feature 1..34: note = Description of Artificial Sequence: Synthetic oligonucleotide
  source 1..34: mol_type = other DNA
gtgactggagttcagacgtgtgctcttccgatct

SEQ ID NO: 17 - DNA, 28 bp, synthetic construct
  misc_feature 1..28: note = Description of Artificial Sequence: Synthetic oligonucleotide
  source 1..28: mol_type = other DNA
acactctttccctacacgacgctcttcc

SEQ ID NO: 18 - RNA, 16 nt, synthetic construct
  misc_feature 1..16: note = Description of Artificial Sequence: Synthetic oligonucleotide
  misc_difference 11..16: note = a, c, u, g, unknown or other
  source 1..16: mol_type = other RNA
  modified_base 2..3: mod_base = OTHER; note = Uracil
  modified_base 8: mod_base = OTHER; note = Uracil
  modified_base 10: mod_base = OTHER; note = Uracil
cttccgatctnnnnnn